European Patent Application EP 4 299 657 A1, published January 3, 2024. Title: Integrated chemical and biological depolymerization of Poly(ethylene terephthalate) for Poly(ethylene terephthalate) upcycling. Applicant: Korea University Research and Business Foundation. The sequence listing filed with the application follows.

SEQUENCE LISTING (4 sequences)

SEQ ID NO: 1 - DNA, 804 bp, Artificial Sequence
  IsPETase_mut
catatgcagaccaatccgtatgcgcgtggcccgaatccgaccgcggcgagcctggaagcgagcgcgggtccgtttaccgtgcgtagctttaccgtgagccgtccgagcggttatggtgcgggtaccgtttactatccgaccaacgcgggtggcaccgtgggtgcgatcgcgattgttccgggttataccgcgcgtcagagcagcatcaaatggtggggtccgcgtctggcgagccacggtttcgtggttatcaccattgacaccaacagcaccctggatcagccggaaagccgtagcagccagcaaatggcggcgctgcgtcaagttgcgagcctgaacggtaccagcagcagcccgatctacggcaaggtggacaccgcgcgtatgggcgttatgggttggagcatgggtggcggtggcagcctgattagcgcggcgaacaacccgagcctgaaagcggcggcgccgcaagcgccgtggcatagcagcaccaacttcagcagcgtgaccgttccgaccctgatctttgcgtgcgagaacgacagcattgcgccggtgaacagcagcgcgctgccgatctacgatagcatgagccgtaacgcgaagcagttcctggaaattaacggtggcagccacagctgcgcgaacagcggtaacagcaaccaagcgctgattggcaagaaaggtgttgcgtggatgaaacgttttatggacaacgatacccgttatagcacctttgcgtgcgaaaatccgaatagcaccgcggtgagcgacttccgtaccgcgaactgcagctaactcgag

SEQ ID NO: 2 - DNA, 1767 bp, Artificial Sequence
  IsMHETase_mut
catatgggtggtggtagcaccccgctgccgctgccgcaacaacaaccgccgcaacaggagccgccgccgccgccggttccgctggcgagccgcgcggcgtgcgaggcgctgaaggatggcaacggtgacatggtgtggccgaacgcggcgaccgtggttgaagttgcggcgtggcgtgatgcggcgccggcgaccgcgagcgcggcggcgctgccggagcactgcgaagtgagcggtgcgatcgcgaagcgtaccggcattgacggttacccgtatgagatcaaatttcgtctgcgtatgccggcggagtggaacggccgtttctttatggaaggtggcagcggtaccaacggtagcctgagcgcggcgaccggtagcatcggtggcggtcagattgcgagcgcgctgagccgtaactttgcgaccattgcgaccgatggcggtcacgacaacgcggtgaacgataacccggatgcgctgggtaccgttgcgttcggtctggacccgcaagcgcgtctggacatgggctacaacagctatgatcaggttacccaagcgggcaaggcggcggttgcgcgtttctacggtcgtgcggcggacaaaagctattttatcggctgcagcgagggcggtcgtgagggtatgatgctgagccagcgtttcccgagccattatgatggtattgtggcgggtgcgccgggttatcaactgccgaaggcgggcattagcggtgcgtggaccacccaaagcctggcgccggcggcggtgggcctggacgcgcaaggtgttccgctgattaacaaaagttttagcgacgcggatctgcacctgctgagccaggcgatcctgggtacctgcgatgcgctggacggcctggcggatggtattgttgacaactatcgtgcgtgccaagcggcgtttgatccggcgaccgcggcgaacccggcgaacggtcaggcgctgcaatgcgttggtgcgaaaaccgcggactgcctgagcccggtgcaggttaccgcgatcaaacgtgcgatggcgggtccggttaacagcgcgggtaccccgctgtacaaccgttgggcgtgggatgcgggtatgagcggtctgagcggtaccacctataaccagggctggcgttccgcgtggctgggtagcttcaacagcagcgcgaacaacgcgcaacgtgtgagcggtttcagcgcgcgtagctggctggttgacttcgcgaccccgccggaaccgatgccgatgacccaggttgcggcgcgtatgatgaagttcgactttgatatcgacccgctgaaaatttgggcgaccagcggccagttcacccaaagcagcatggattggcatggtgcgaccagcaccgatctggcggcgtttcgtgaccgtggcggtaaaatgatcctgtatcatggtatgagcgatgcggcgttcagcgcgctggataccgcggactactatgaacgtctgggtgcggcgatgccgggtgcggcgggtttcgcgcgtctgtttctggttccgggtatgaaccattgcagcggcggtccgggtaccgatcgttttgacatgctgaccccgctggttgcgtgggttgagcgtggtgaagcgccggatcaaatcagcgcgtggagcggtaccccgggttacttcggtgtggcggcgcgtacccgtccgctgtgcccgtatccgcaaattgcgcgttacaagggcagcggtgacatcaataccgaagcgaactttgcgtgcgcggcgccgccgtaactcgag

SEQ ID NO: 3 - DNA, 801 bp, Artificial Sequence
  IsMHETase_wt
catatgcaaacaaacccctatgctcggggccccaaccctacagccgcttcattggaagctagcgccggtccgtttaccgtacgctcatttacggtgagccggcctagtggttatggtgcggggaccgtgtattaccctacaaatgccggcggtactgtgggcgcaattgcgatcgtgccgggctataccgcgcgtcagtcgtctattaaatggtggggcccacgtttagcatcacacggatttgtagtcattactattgacaccaacagtacgcttgatcagccgtcatctcgatccagtcagcagatggccgcgctgagacaagttgcgtctctcaatggcacgagcagctcaccgatatacggtaaagttgatactgcacgtatgggggttatgggatggtccatgggcggtggcggctctctaatcagtgccgcgaataatccgtcgctgaaagctgcagcaccgcaggccccatgggatagttcgactaacttctcatcggtcaccgtaccaacgctgatatttgcttgcgaaaatgacagtattgccccggtcaattcgtccgctttaccgatctatgatagcatgtcacgcaatgcgaagcaatttttggagattaatggtggatcccattcttgtgctaatagcggaaatagcaatcaagcgcttatcggcaagaaaggcgttgcatggatgaaacgcttcatggataatgatacgaggtactccacattcgcctgtgaaaatccaaacagcacacgagtttctgactttcgtaccgccaattgcagtctcgag

SEQ ID NO: 4 - DNA, 1767 bp, Artificial Sequence
  IsMHETase_wt
catatgggtggtggtagcaccccgctgccgctgccgcaacaacaaccgccgcaacaggagccgccgccgccgccggttccgctggcgagccgcgcggcgtgcgaggcgctgaaggatggcaacggtgacatggtgtggccgaacgcggcgaccgtggttgaagttgcggcgtggcgtgatgcggcgccggcgaccgcgagcgcggcggcgctgccggagcactgcgaagtgagcggtgcgatcgcgaagcgtaccggcattgacggttacccgtatgagatcaaatttcgtctgcgtatgccggcggagtggaacggccgtttctttatggaaggtggcagcggtaccaacggtagcctgagcgcggcgaccggtagcatcggtggcggtcagattgcgagcgcgctgagccgtaactttgcgaccattgcgaccgatggcggtcacgacaacgcggtgaacgataacccggatgcgctgggtaccgttgcgttcggtctggacccgcaagcgcgtctggacatgggctacaacagctatgatcaggttacccaagcgggcaaggcggcggttgcgcgtttctacggtcgtgcggcggacaaaagctattttatcggctgcagcgagggcggtcgtgagggtatgatgctgagccagcgtttcccgagccattatgatggtattgtggcgggtgcgccgggttatcaactgccgaaggcgggcattagcggtgcgtggaccacccaaagcctggcgccggcggcggtgggcctggacgcgcaaggtgttccgctgattaacaaaagttttagcgacgcggatctgcacctgctgagccaggcgatcctgggtacctgcgatgcgctggacggcctggcggatggtattgttgacaactatcgtgcgtgccaagcggcgtttgatccggcgaccgcggcgaacccggcgaacggtcaggcgctgcaatgcgttggtgcgaaaaccgcggactgcctgagcccggtgcaggttaccgcgatcaaacgtgcgatggcgggtccggttaacagcgcgggtaccccgctgtacaaccgttgggcgtgggatgcgggtatgagcggtctgagcggtaccacctataaccagggctggcgttcctggtggctgggtagcttcaacagcagcgcgaacaacgcgcaacgtgtgagcggtttcagcgcgcgtagctggctggttgacttcgcgaccccgccggaaccgatgccgatgacccaggttgcggcgcgtatgatgaagttcgactttgatatcgacccgctgaaaatttgggcgaccagcggccagttcacccaaagcagcatggattggcatggtgcgaccagcaccgatctggcggcgtttcgtgaccgtggcggtaaaatgatcctgtatcatggtatgagcgatgcggcgttcagcgcgctggataccgcggactactatgaacgtctgggtgcggcgatgccgggtgcggcgggtttcgcgcgtctgtttctggttccgggtatgaaccattgcagcggcggtccgggtaccgatcgttttgacatgctgaccccgctggttgcgtgggttgagcgtggtgaagcgccggatcaaatcagcgcgtggagcggtaccccgggttacttcggtgtggcggcgcgtacccgtccgctgtgcccgtatccgcaaattgcgcgttacaagggcagcggtgacatcaataccgaagcgaactttgcgtgcgcggcgccgccgtaactcgag